European Patent Specification EP 3 881 326 B1, published April 5, 2023. Title: BIOLOGICAL SEQUENCE INFORMATION HANDLING. Applicant: Biostrand BVBA BioKey BVBA. Application EPPCTNYK. The sequence listing filed with the application follows.

SEQUENCE LISTING (10 sequences)

SEQ ID NO: 1 - protein, 7 aa, Unknown
  Unknown
MCMHNQA

SEQ ID NO: 2 - protein, 6 aa, Unknown
  Unknown
MCMHNQ

SEQ ID NO: 3 - protein, 25 aa, Unknown
  Unknown
AVFPSIVGRPRHQGVMVGMGQKDSY

SEQ ID NO: 4 - protein, 11 aa, Unknown
  Unknown
IVGRPRHQGVM

SEQ ID NO: 5 - protein, 11 aa, Unknown
  Unknown
FAGDDAPRAVF

SEQ ID NO: 6 - protein, 11 aa, Unknown
  Unknown
IVGRPRHQGVM

SEQ ID NO: 7 - protein, 11 aa, Unknown
  Unknown
IITNWDDMEKI

SEQ ID NO: 8 - protein, 11 aa, Unknown
  Unknown
IMFETFNVPAM

SEQ ID NO: 9 - protein, 11 aa, Unknown
  Unknown
IKEKLCYVALD

SEQ ID NO: 10 - protein, 11 aa, Unknown
  Unknown
IGMESAGIHET